European Patent Specification EP 3 229 611 B1, published March 26, 2025. Title: COMPOUNDS THAT MODULATE FATTY ACID RECEPTOR ACTIVITY AND PET FOOD PRODUCTS CONTAINING THE SAME. Applicant: MARS, INCORPORATED. The sequence listing filed with the application follows.

SEQUENCE LISTING (1 sequence)

SEQ ID NO: 1 - protein, 361 aa, Felis catus
MSPECAQAAGTGSPRSLERANRTRFPFFSDVKGDHRLVLTAVETVVLALIFAVSLLGNVCALVLVARRRRRGTTACLVLNLFCADLLFTSAIPPVLAVRWTEAWLLGPVACHLLFYVMSLSGSVTILTLAAVSLERMVCIVRLQRGVRGLGRRARAALLALIWGYSALAALPLCVFFQVVPQRLSGRDQEIPICTLSWPSIAGEISWDVSFVTLNFLMPGLLIVISYSKILQITKASRKRLTVNLASSESHHIRVSQQDFRLFRTLFLLMISFFIMWSPIIITILLILIQNFKQDLVIWPSLFFWVVAFTFANSALNPILYNMSLFRNEWRKIFHCFFYPEKGAMFTDTSVRRNDLSVISN